European Patent Specification EP 3 851 537 B1, published December 27, 2023. Title: TREATMENT OF HYPERBILIRUBINEMIA. Applicant: GENETHON et al. The sequence listing filed with the application follows.

SEQUENCE LISTING (11 sequences)

SEQ ID NO: 1 - DNA, 1602 bp, homo sapiens
atggctgtggagtcccagggcggacgcccacttgtcctgggcctgctgctgtgtgtgctgggcccagtggtgtcccatgctgggaagatactgttgatcccagtggatggcagccactggctgagcatgcttggggccatccagcagctgcagcagaggggacatgaaatagttgtcctagcacctgacgcctcgttgtacatcagagacggagcattttacaccttgaagacgtaccctgtgccattccaaagggaggatgtgaaagagtcttttgttagtctcgggcataatgtttttgagaatgattctttcctgcagcgtgtgatcaaaacatacaagaaaataaaaaaggactctgctatgcttttgtctggctgttcccacttactgcacaacaaggagctcatggcctccctggcagaaagcagctttgatgtcatgctgacggaccctttccttccttgcagccccatcgtggcccagtacctgtctctgcccactgtattcttcttgcatgcactgccatgcagcctggaatttgaggctacccagtgccccaacccattctcctacgtgcccaggcctctctcctctcattcagatcacatgaccttcctgcagcgggtgaagaacatgctcattgccttttcacagaactttctgtgcgacgtggtttattccccgtatgcaacccttgcctcagaattccttcagagagaggtgactgtccaggacctattgagctctgcatctgtctggctgtttagaagtgactttgtgaaggattaccctaggcccatcatgcccaatatggtttttgttggtggaatcaactgccttcaccaaaatccactatcccaggaatttgaagcctacattaatgcttctggagaacatggaattgtggttttctctttgggatcaatggtctcagaaattccagagaagaaagctatggcaattgctgatgctttgggcaaaatccctcagacagtcctgtggcggtacactggaacccgaccatcgaatcttgcgaacaacacgatacttgttaagtggctaccccaaaacgatctgcttggtcacccgatgacccgtgcctttatcacccatgctggttcccatggtgtttatgaaagcatatgcaatggcgttcccatggtgatgatgcccttgtttggtgatcagatggacaatgcaaagcgcatggagactaagggagctggagtgaccctgaatgttctggaaatgacttctgaagatttagaaaatgctctaaaagcagtcatcaatgacaaaagttacaaggagaacatcatgcgcctctccagccttcacaaggaccgcccggtggagccgctggacctggccgtgttctgggtggagtttgtgatgaggcacaagggcgcgccacacctgcgccccgcagcccacgacctcacctggtaccagtaccattccttggacgtgattggtttcctcttggccgtcgtgctgacagtggccttcatcacctttaaatgttgtgcttatggctaccggaaatgcttggggaaaaaagggcgagttaagaaagcccacaaatccaagacccattga

SEQ ID NO: 2 - DNA, 1602 bp, artificial
  optimized UGT1A1 v2.1
atggctgtggaatcacaaggaggtagaccactggttctcggacttttgctttgcgtgctggggcccgtggtgtcgcatgccggaaagatcctgctgatcccggtggatggatcacactggctgtccatgctgggtgccatccaacagctccagcagcggggccacgaaattgtggtcctggccccggacgcttccctgtatattcgggacggagcgttctacactctcaagacctaccctgtccccttccaaagggaggacgtgaaggaaagctttgtgtcgctggggcataatgtgttcgagaacgacagcttcctccaaagggttattaaaacctacaagaagatcaaaaaggattcggccatgctcctttccggatgttcacacctgttgcataacaaggaattgatggccagcctggcagaatccagctttgacgtcatgcttactgacccgttcttgccttgctccccgattgtggcccaatacctgtcgctcccaaccgtgttcttcctgcacgccttgccttgttcgctggaattcgaagcgactcagtgtcccaatccgttctcctacgtcccgcgcccgctttcaagccattcggatcacatgactttcctccagcgcgtcaagaacatgctcattgcgttcagccagaactttctgtgcgacgtggtttactcaccttacgctaccttggcttctgagttcctgcagagagaagtgactgtgcaagatctgctgtcctcagcgtccgtttggttgttccggtctgacttcgtcaaggactacccgcgcccgatcatgccgaatatggtctttgtgggcggtatcaactgcctgcatcaaaacccactgagccaggagtttgaggcgtacatcaacgcctcgggagagcatggaatcgtggtgttctccctcggttccatggtgtccgagatcccggaaaagaaggcaatggccatcgcagatgccctgggcaaaatcccgcagaccgtgctctggcgctacacgggtactcggcctagcaatttggcaaacaacaccatcctggtgaaatggctgccgcagaacgacctcctgggccacccaatgactcgcgctttcattacccatgcgggctcgcacggagtctacgaatccatctgcaatggagtcccgatggtgatgatgccacttttcggagatcagatggataatgcaaaaagaatggaaaccaagggggccggagtgacgctgaacgtgcttgaaatgacctcggaagatctggagaacgctctcaaagcggtgatcaacgacaagtcctacaaggaaaacatcatgcgcctgagctccctccacaaggaccgaccagtggaaccgctggacctcgcggtcttttgggtggagttcgtgatgaggcacaagggcgccccccacctcagacccgcagctcatgacctcacttggtaccagtaccattcgctggatgtcatcggctttctcctggcggtcgtgctcaccgtggcgttcatcaccttcaagtgctgcgcctacggatatcgcaaatgcttggggaagaaaggacgggtgaagaaggcacacaagtcaaagacgcactga

SEQ ID NO: 3 - DNA, 1602 bp, artificial
  optimized UGT1A1 v3
atggccgtggaatctcagggcggcagacctctggtgctgggcctgctgctgtgtgtgctgggacctgtggtgtctcacgccggcaagatcctgctgatccccgtggatggcagccactggctgtctatgctgggcgccattcagcagctgcagcagaggggccacgagatcgtggtgctggcccctgatgccagcctgtacatcagagatggcgccttctacaccctgaaaacctaccccgtgcccttccagcgcgaggacgtgaaagaaagcttcgtgtccctgggccacaacgtgttcgagaacgacagcttcctgcagagagtgatcaagacctacaagaagatcaagaaagacagcgccatgctgctgagcggctgctcccatctgctgcacaacaaagaactgatggcctccctggccgagagcagcttcgacgtgatgctgaccgacccattcctgccctgcagccctatcgtggcccagtacctgagcctgcctaccgtgttcttcctgcacgccctgccttgctccctggaattcgaggccacccagtgccccaaccccttcagctacgtgcccagaccactgagcagccacagcgaccacatgacctttctgcagcgcgtgaagaacatgctgatcgccttcagccagaacttcctgtgcgacgtggtgtacagcccctacgctaccctggccagcgaattcctgcagcgggaagtgaccgtgcaggacctgctgtctagcgccagcgtgtggctgttccgcagcgacttcgtgaaggactaccccagacccatcatgcccaacatggtgttcgtgggcggcatcaactgcctgcaccagaaccccctgagccaggaatttgaggcctacatcaacgccagcggcgagcacggcatcgtggtgtttagcctgggcagcatggtgtccgagatccccgagaaaaaggccatggctatcgccgacgccctgggaaagatcccccagacagtgctgtggcggtacaccggcaccagacccagcaacctggccaacaacaccatcctcgtgaaatggctgccccagaacgacctgctgggccaccctatgacccgggcctttatcacacacgccggctcccatggcgtgtacgagagcatctgcaacggcgtgcccatggtcatgatgcccctgttcggcgaccagatggacaacgccaagcggatggaaacaaagggcgctggcgtgaccctgaacgtgctggaaatgaccagcgaggacctggaaaacgccctgaaggccgtgatcaacgacaagagctacaaagaaaacatcatgcggctgtccagcctgcacaaggacagacccgtggaacccctggacctggccgtgttctgggtggaattcgtgatgcggcacaagggcgctccccatctgaggcctgcagctcacgacctgacctggtatcagtaccacagcctggacgtgatcggcttcctgctggcagtggtgctgaccgtggccttcatcaccttcaagtgctgcgcctacggctaccggaagtgcctgggcaagaaaggcagagtgaagaaggcccacaagagcaagacccactga

SEQ ID NO: 4 - DNA, 397 bp, homo sapiens
gatcttgctaccagtggaacagccactaaggattctgcagtgagagcagagggccagctaagtggtactctcccagagactgtctgactcacgccaccccctccaccttggacacaggacgctgtggtttctgagccaggtacaatgactcctttcggtaagtgcagtggaagctgtacactgcccaggcaaagcgtccgggcagcgtaggcgggcgactcagatcccagccagtggacttagcccctgtttgctcctccgataactggggtgaccttggttaatattcaccagcagcctcccccgttgcccctctggatccactgcttaaatacggacgaggacagggccctgtctcctcagcttcaggcaccaccactgacctgggacagtgaat

SEQ ID NO: 5 - DNA, 441 bp, artificial
  HBB2 intron
gtacacatattgaccaaatcagggtaattttgcatttgtaattttaaaaaatgctttcttcttttaatatacttttttgtttatcttatttctaatactttccctaatctctttctttcagggcaataatgatacaatgtatcatgcctctttgcaccattctaaagaataacagtgataatttctgggttaaggcaatagcaatatttctgcatataaatatttctgcatataaattgtaactgatgtaagaggtttcatattgctaatagcagctacaatccagctaccattctgcttttattttatggttgggataaggctggattattctgagtccaagctaggcccttttgctaatcatgttcatacctcttatcttcctcccacagctcctgggcaacgtgctggtctgtgtgctggcccatcactttggcaaag

SEQ ID NO: 6 - DNA, 441 bp, artificial
  modified HBB2 intron
gtacacatattgaccaaatcagggtaattttgcatttgtaattttaaaaaatgctttcttcttttaatatacttttttgtttatcttatttctaatactttccctaatctctttctttcagggcaataatgatacaatgtatcatgcctctttgcaccattctaaagaataacagtgataatttctgggttaaggcaatagcaatatttctgcatataaatatttctgcatataaattgtaactgatgtaagaggtttcatattgctaatagcagctacaatccagctaccattctgcttttattttctggttgggataaggctggattattctgagtccaagctaggcccttttgctaatcttgttcatacctcttatcttcctcccacagctcctgggcaacctgctggtctctctgctggcccatcactttggcaaag

SEQ ID NO: 7 - DNA, 1438 bp, artificial
  FIX intron
ggtttgtttccttttttaaaatacattgagtatgcttgccttttagatatagaaatatctgatgctgtcttcttcactaaattttgattacatgatttgacagcaatattgaagagtctaacagccagcacgcaggttggtaagtactggttctttgttagctaggttttcttcttcttcatttttaaaactaaatagatcgacaatgcttatgatgcatttatgtttaataaacactgttcagttcatgatttggtcatgtaattcctgttagaaaacattcatctccttggtttaaaaaaattaaaagtgggaaaacaaagaaatagcagaatatagtgaaaaaaaataaccacattatttttgtttggacttaccactttgaaatcaaaatgggaaacaaaagcacaaacaatggccttatttacacaaaaagtctgattttaagatatatgacatttcaaggtttcagaagtatgtaatgaggtgtgtctctaattttttaaattatatatcttcaatttaaagttttagttaaaacataaagattaacctttcattagcaagctgttagttatcaccaacgcttttcatggattaggaaaaaatcattttgtctctatgtcaaacatcttggagttgatatttggggaaacacaatactcagttgagttccctaggggagaaaagcacgcttaagaattgacataaagagtaggaagttagctaatgcaacatatatcactttgttttttcacaactacagtgactttatgtatttcccagaggaaggcatacagggaagaaattatcccatttggacaaacagcatgttctcacaggaagcatttatcacacttacttgtcaactttctagaatcaaatctagtagctgacagtaccaggatcaggggtgccaaccctaagcacccccagaaagctgactggccctgtggttcccactccagacatgatgtcagctgtgaaatcgacgtcgctggaccataattaggcttctgttcttcaggagacatttgttcaaagtcatttgggcaaccatattctgaaaacagcccagccagggtgatggatcactttgcaaagatcctcaatgagctattttcaagtgatgacaaagtgtgaagttaaccgctcatttgagaactttctttttcatccaaagtaaattcaaatatgattagaaatctgaccttttattactggaattctcttgactaaaagtaaaattgaattttaattcctaaatctccatgtgtatacagtactgtgggaacatcacagattttggctccatgccctaaagagaaattggctttcagattatttggattaaaaacaaagactttcttaagagatgtaaaattttcatgatgttttcttttttgctaaaactaaagaattattcttttacatttca

SEQ ID NO: 8 - DNA, 1438 bp, artificial
  modified FIX intron
ggtttgtttccttttttaaaatacattgagtatgcttgccttttagatatagaaatatctgatgctgtcttcttcactaaattttgattacatgatttgacagcaatattgaagagtctaacagccagcacgcaggttggtaagtactggttctttgttagctaggttttcttcttcttcatttttaaaactaaatagatcgacattgcttttgttgcatttatgtttaataaacactgttcagttcatgatttggtcatgtaattcctgttagaaaacattcatctccttggtttaaaaaaattaaaagtgggaaaacaaagaaatagcagaatatagtgaaaaaaaataaccacattatttttgtttggacttaccactttgaaatcaaattgggaaacaaaagcacaaacaatggccttatttacacaaaaagtctgattttaagatatatgacatttcaaggtttcagaagtatgtaatgaggtgtgtctctaattttttaaattatatatcttcaatttaaagttttagttaaaacataaagattaacctttcattagcaagctgttagttatcaccaacgcttttcatggattaggaaaaaatcattttgtctctttgtcaaacatcttggagttgatatttggggaaacacaatactcagttgagttccctaggggagaaaagcacgcttaagaattgacataaagagtaggaagttagctattgcaacatatatcactttgttttttcacaactacagtgactttttgtatttcccagaggaaggcatacagggaagaaattatcccatttggacaaacagcttgttctcacaggaagcatttatcacacttacttgtcaactttctagaatcaaatctagtagctgacagtaccaggatcaggggtgccaaccctaagcacccccagaaagctgactggccctgtggttcccactccagacatgatgtcagctgtgaaatcgacgtcgctggaccataattaggcttctgttcttcaggagacatttgttcaaagtcatttgggcaaccatattctgaaaacagcccagccagggtgttggatcactttgcaaagatcctcattgagctattttcaagtgttgacaaagtgtgaagttaaccgctcatttgagaactttctttttcatccaaagtaaattcaaatatgattagaaatctgaccttttattactggaattctcttgactaaaagtaaaattgaattttaattcctaaatctccatgtgtatacagtactgtgggaacatcacagattttggctccatgccctaaagagaaattggctttcagattatttggattaaaaacaaagactttcttaagagatgtaaaattttcttgttgttttcttttttgctaaaactaaagaattattcttttacatttca

SEQ ID NO: 9 - DNA, 881 bp, artificial
  chicken beta-globin intron
gcgggagtcgctgcgttgccttcgccccgtgccccgctccgccgccgcctcgcgccgcccgccccggctctgactgaccgcgttactcccacaggtgagcgggcgggacggcccttctcctccgggctgtaattagcgcttggtttaatgacggcttgtttcttttctgtggctgcgtgaaagccttgaggggctccgggagggccctttgtgcggggggagcggctcggggggtgcgtgcgtgtgtgtgtgcgtggggagcgccgcgtgcggctccgcgctgcccggcggctgtgagcgctgcgggcgcggcgcggggctttgtgcgctccgcagtgtgcgcgaggggagcgcggccgggggcggtgccccgcggtgcggggggggctgcgaggggaacaaaggctgcgtgcggggtgtgtgcgtgggggggtgagcagggggtgtgggcgcgtcggtcgggctgcaaccccccctgcacccccctccccgagttgctgagcacggcccggcttcgggtgcggggctccgtacggggcgtggcgcggggctcgccgtgccgggcggggggtggcggcaggtgggggtgccgggcggggcggggccgcctcgggccggggagggctcgggggaggggcgcggcggcccccggagcgccggcggctgtcgaggcgcggcgagccgcagccattgccttttatggtaatcgtgcgagagggcgcagggacttcctttgtcccaaatctgtgcggagccgaaatctgggaggcgccgccgcaccccctctagcgggcgcggggcgaagcggtgcggcgccggcaggaaggaaatgggcggggagggccttcgtgcgtcgccgcgccgccgtccccttctccctc

SEQ ID NO: 10 - DNA, 881 bp, artificial
  optimized chicken beta-globin intron
gcgggagtcgctgcgttgccttcgccccgtgccccgctccgccgccgcctcgcgccgcccgccccggctctgactgaccgcgttactcccacaggtgagcgggcgggacggcccttctcctccgggctgtaattagcgcttggtttaatgacggcttgtttcttttctgtggctgcgtgaaagccttgaggggctccgggagggccctttgtgcggggggagcggctcggggggtgcgtgcgtgtgtgtgtgcgtggggagcgccgcgtgcggctccgcgctgcccggcggctgtgagcgctgcgggcgcggcgcggggctttgtgcgctccgcagtgtgcgcgaggggagcgcggccgggggcggtgccccgcggtgcggggggggctgcgaggggaacaaaggctgcgtgcggggtgtgtgcgtgggggggtgagcagggggtgtgggcgcgtcggtcgggctgcaaccccccctgcacccccctccccgagttgctgagcacggcccggcttcgggtgcggggctccgtacggggcgtggcgcggggctcgccgtgccgggcggggggtggcggcaggtgggggtgccgggcggggcggggccgcctcgggccggggagggctcgggggaggggcgcggcggcccccggagcgccggcggctgtcgaggcgcggcgagccgcagccattgccttttttggtaatcgtgcgagagggcgcagggacttcctttgtcccaaatctgtgcggagccgaaatctgggaggcgccgccgcaccccctctagcgggcgcggggcgaagcggtgcggcgccggcaggaaggaattgggcggggagggccttcgtgcgtcgccgcgccgccgtccccttctccctc

SEQ ID NO: 11 - DNA, 322 bp, artificial
  ApoE control region
aaggctcagaggcacacaggagtttctgggctcaccctgcccccttccaacccctcagttcccatcctccagcagctgtttgtgtgctgcctctgaagtccacactgaacaaacttcagcctactcatgtccctaaaatgggcaaacattgcaagcagcaaacagcaaacacacagccctccctgcctgctgaccttggagctggggcagaggtcagagacctctctgggcccatgccacctccaacatccactcgaccccttggaatttcggtggagaggagcagaggttgtcctggcgtggtttaggtagtgtgagaggg